European Patent Application EP 4 410 965 A1, published August 7, 2024. Title: Ｔ細胞の製造方法. Applicant: 国立大学法人京都大学. The sequence listing filed with the application follows.

SEQUENCE LISTING (8 sequences)

SEQ ID NO: 1 - DNA, 1191 bp, Homo sapiens
  source 1..1191: mol_type = other DNA
atgcccaaccccaggcctggcaagccctcggccccttccttggcccttggcccatccccaggagcctcgcccagctggagggctgcacccaaagcctcagacctgctgggggcccggggcccagggggaaccttccagggccgagatcttcgaggcggggcccatgcctcctcttcttccttgaaccccatgccaccatcgcagctgcagctctcaacggtggatgcccacgcccggacccctgtgctgcaggtgcaccccctggagagcccagccatgatcagcctcacaccacccaccaccgccactggggtcttctccctcaaggcccggcctggcctcccacctgggatcaacgtggccagcctggaatgggtgtccagggagccggcactgctctgcaccttcccaaatcccagtgcacccaggaaggacagcaccctttcggctgtgccccagagctcctacccactgctggcaaatggtgtctgcaagtggcccggatgtgagaaggtcttcgaagagccagaggacttcctcaagcactgccaggcggaccatcttctggatgagaagggcagggcacaatgtctcctccagagagagatggtacagtctctggagcagcagctggtgctggagaaggagaagctgagtgccatgcaggcccacctggctgggaaaatggcactgaccaaggcttcatctgtggcatcatccgacaagggctcctgctgcatcgtagctgctggcagccaaggccctgtcgtcccagcctggtctggcccccgggaggcccctgacagcctgtttgctgtccggaggcacctgtggggtagccatggaaacagcacattcccagagttcctccacaacatggactacttcaagttccacaacatgcgaccccctttcacctacgccacgctcatccgctgggccatcctggaggctccagagaagcagcggacactcaatgagatctaccactggttcacacgcatgtttgccttcttcagaaaccatcctgccacctggaagaacgccatccgccacaacctgagtctgcacaagtgctttgtgcgggtggagagcgagaagggggctgtgtggaccgtggatgagctggagttccgcaagaaacggagccagaggcccagcaggtgttccaaccctacacctggcccctga

SEQ ID NO: 2 - DNA, 1296 bp, Homo sapiens
  source 1..1296: mol_type = other DNA
atgcccaaccccaggcctggcaagccctcggccccttccttggcccttggcccatccccaggagcctcgcccagctggagggctgcacccaaagcctcagacctgctgggggcccggggcccagggggaaccttccagggccgagatcttcgaggcggggcccatgcctcctcttcttccttgaaccccatgccaccatcgcagctgcagctgcccacactgcccctagtcatggtggcaccctccggggcacggctgggccccttgccccacttacaggcactcctccaggacaggccacatttcatgcaccagctctcaacggtggatgcccacgcccggacccctgtgctgcaggtgcaccccctggagagcccagccatgatcagcctcacaccacccaccaccgccactggggtcttctccctcaaggcccggcctggcctcccacctgggatcaacgtggccagcctggaatgggtgtccagggagccggcactgctctgcaccttcccaaatcccagtgcacccaggaaggacagcaccctttcggctgtgccccagagctcctacccactgctggcaaatggtgtctgcaagtggcccggatgtgagaaggtcttcgaagagccagaggacttcctcaagcactgccaggcggaccatcttctggatgagaagggcagggcacaatgtctcctccagagagagatggtacagtctctggagcagcagctggtgctggagaaggagaagctgagtgccatgcaggcccacctggctgggaaaatggcactgaccaaggcttcatctgtggcatcatccgacaagggctcctgctgcatcgtagctgctggcagccaaggccctgtcgtcccagcctggtctggcccccgggaggcccctgacagcctgtttgctgtccggaggcacctgtggggtagccatggaaacagcacattcccagagttcctccacaacatggactacttcaagttccacaacatgcgaccccctttcacctacgccacgctcatccgctgggccatcctggaggctccagagaagcagcggacactcaatgagatctaccactggttcacacgcatgtttgccttcttcagaaaccatcctgccacctggaagaacgccatccgccacaacctgagtctgcacaagtgctttgtgcgggtggagagcgagaagggggctgtgtggaccgtggatgagctggagttccgcaagaaacggagccagaggcccagcaggtgttccaaccctacacctggcccctga

SEQ ID NO: 3 - protein, 396 aa, Homo sapiens
MPNPRPGKPSAPSLALGPSPGASPSWRAAPKASDLLGARGPGGTFQGRDLRGGAHASSSSLNPMPPSQLQLSTVDAHARTPVLQVHPLESPAMISLTPPTTATGVFSLKARPGLPPGINVASLEWVSREPALLCTFPNPSAPRKDSTLSAVPQSSYPLLANGVCKWPGCEKVFEEPEDFLKHCQADHLLDEKGRAQCLLQREMVQSLEQQLVLEKEKLSAMQAHLAGKMALTKASSVASSDKGSCCIVAAGSQGPVVPAWSGPREAPDSLFAVRRHLWGSHGNSTFPEFLHNMDYFKFHNMRPPFTYATLIRWAILEAPEKQRTLNEIYHWFTRMFAFFRNHPATWKNAIRHNLSLHKCFVRVESEKGAVWTVDELEFRKKRSQRPSRCSNPTPGP

SEQ ID NO: 4 - protein, 431 aa, Homo sapiens
MPNPRPGKPSAPSLALGPSPGASPSWRAAPKASDLLGARGPGGTFQGRDLRGGAHASSSSLNPMPPSQLQLPTLPLVMVAPSGARLGPLPHLQALLQDRPHFMHQLSTVDAHARTPVLQVHPLESPAMISLTPPTTATGVFSLKARPGLPPGINVASLEWVSREPALLCTFPNPSAPRKDSTLSAVPQSSYPLLANGVCKWPGCEKVFEEPEDFLKHCQADHLLDEKGRAQCLLQREMVQSLEQQLVLEKEKLSAMQAHLAGKMALTKASSVASSDKGSCCIVAAGSQGPVVPAWSGPREAPDSLFAVRRHLWGSHGNSTFPEFLHNMDYFKFHNMRPPFTYATLIRWAILEAPEKQRTLNEIYHWFTRMFAFFRNHPATWKNAIRHNLSLHKCFVRVESEKGAVWTVDELEFRKKRSQRPSRCSNPTPGP

SEQ ID NO: 5 - DNA, 238 bp, Homo sapiens
  source 1..238: mol_type = other DNA
taggttagtctttttttctgtggcttctgtctctggttttgtgcttagaaagtcctttcctacttgaaaatgagataaatgttcacctatgttggcttctagtctcttttatggcttcattttttccatttactatagaggttaagagtgtgggtactggagccagactgtctgggacaaacccagcgtcaccccaagccctatgtgtgatttttagccaggcacttaacctctccat

SEQ ID NO: 6 - DNA, 360 bp, Homo sapiens
  source 1..360: mol_type = other DNA
ccaagaagggccaggtcttcagagctaggggcttgtcatagtggccagatggacatcacctaccacatccaccagcacccatgtcaccccacctgggccaagcctgctgcaggacagggcagccagttctcggaacgaaacctgtggggtggggtatctgccctcttctcttcctccgtggtgtcgatgaagcccggcgcatccggccgccatgacgtcaatggcggaaaaatctgggcaagtcgggggctgtgacaacagggcccagatgcagaccccgatatgaaaacataatctgtgtcccagaaacatcccccattcagcttctgagaaacccagtcagaaagggacgtcccaaca

SEQ ID NO: 7 - DNA, 218 bp, Homo sapiens
  source 1..218: mol_type = other DNA
gaggccctgggcccaggatggggcaggcagggtggggtacctggacctacaggtgccgacctttactgtggcactgggcgggaggggggctggctggggcacaggaagtggtttctgggtcccaggcaagtctgtgacttatgcagatgttgcagggccaagaaaatccccacctgccaggcctcagagattggaggctctccccgacctcccaatcc

SEQ ID NO: 8 - DNA, 383 bp, Homo sapiens
  source 1..383: mol_type = other DNA
tcccatccacacatagagcttcagattctctttctttccccagagaccctcaaatatcctctcactcacagaatggtgtctctgcctgcctcgggttggccctgtgatttattttagttcttttcccttgttttttttttttcaaactctatacacttttgttttaaaaactgtggtttctcatgagccctattatctcattgatacctctcacctctgtggtgaggggaagaaatcatattttcagatgactcgtaaagggcaaagaaaaaaacccaaaatttcaaaatttccgtttaagtctcataatcaagaaaaggagaaacacagagagagagaaaaaaaaaactatgagaacccctccccaccccgtgattatcagc